European Patent Application EP 4 450 621 A1, published October 23, 2024. Title: 新規プロモーター. Applicant: 花王株式会社. The sequence listing filed with the application follows.

SEQUENCE LISTING (169 sequences)

SEQ ID NO: 1 - DNA, 613 bp, Corynebacterium glutamicum
  source 1..613: mol_type = genomic DNA
ctcaacatgcgcgaaaatggcggtgaccaggaccttatccagcgcctcgctgctgatgagcgcctcccaatgagcgaagctgaccttgaggcagcgctggctgaccgccacgccttcatcggtgccgctgagtcccaggtctcccgtgtgctcgaccgcattcaggtgcttgtcgacgcccaccccggcgccgcagactaccgaccaggtgagattctttaaaggtttttaacggcgttcacgcgggtttaccgctggatcgcagtgagaaaatggggcctcgagccccattttttgtacccaaagcaactgtgtagctcgaattacgggtccagtgaaggttccgaaaggtgtcttttaggtgtcttaaaaacaacattggtgggcctgaaaacttcaaaaattggccattttggaaaaaaatttaataatttttttacgatgaataaaattacattgcccttaaaggtatctaaatgacacttattaaacggtgttcaaaaatggcccagtttttgacgatggggttgcgggcaaggggcgttatgagccacacttgagtcatcccagtcagacagcaagagtctggcgaacaacagaaagagagatcaca

SEQ ID NO: 2 - DNA, 117 bp, Corynebacterium glutamicum
  source 1..117: mol_type = genomic DNA
atgacctctgtattcgatatcatccagtccatcttcgacggcgttcacggcctcgttggctccatcttcgctggcgcacagggcgtcttcgactccatcgttaccgcttcttcctag

SEQ ID NO: 3 - protein, 38 aa, Corynebacterium glutamicum
MTSVFDIIQSIFDGVHGLVGSIFAGAQGVFDSIVTASS

SEQ ID NO: 4 - DNA, 22 bp, synthetic construct
  source 1..22: mol_type = other DNA
cctgcaggtacgtattacagaa

SEQ ID NO: 5 - DNA, 16 bp, synthetic construct
  source 1..16: mol_type = other DNA
atgcgcactcaggtgg

SEQ ID NO: 6 - DNA, 35 bp, synthetic construct
  source 1..35: mol_type = other DNA
atacgtacctgcaggctcaacatgcgcgaaaatgg

SEQ ID NO: 7 - DNA, 38 bp, synthetic construct
  source 1..38: mol_type = other DNA
cacctgagtgcgcattgtgatctctctttctgttgttc

SEQ ID NO: 8 - DNA, 27 bp, synthetic construct
  source 1..27: mol_type = other DNA
cattgcccttaaaggtatctaaatgac

SEQ ID NO: 9 - DNA, 17 bp, synthetic construct
  source 1..17: mol_type = other DNA
cgagtggcagtcctacg

SEQ ID NO: 10 - DNA, 20 bp, synthetic construct
  source 1..20: mol_type = other DNA
atgcgcactcaggtggctat

SEQ ID NO: 11 - DNA, 20 bp, synthetic construct
  source 1..20: mol_type = other DNA
cctgcaggtacgtattacag

SEQ ID NO: 12 - DNA, 294 bp, synthetic construct
  source 1..294: mol_type = other DNA; note = PL13 promoter
ggcgcttcatgtcaacaatctttaacgttttcaagttcacaagtcgtgttcaaatggtgacaagattggacactgtgctgaattggcaccaagccctcataaatgatagatctaaatcgaatatcaatatatggtctgtttattggaacgcgtcccagtggctgagacgcatccgctaaagccccaggaaccctgtgcagaaagaacaaataatcgtgaattttggcagcaacagcggggcctggtataattgaaaacgtgcaaaagcatagattattggaggagatcaaaaca

SEQ ID NO: 13 - DNA, 35 bp, synthetic construct
  source 1..35: mol_type = other DNA
atacgtacctgcaggggcgcttcatgtcaacaatc

SEQ ID NO: 14 - DNA, 42 bp, synthetic construct
  source 1..42: mol_type = other DNA
cacctgagtgcgcattgttttgatctcctccaataatctatg

SEQ ID NO: 15 - DNA, 21 bp, synthetic construct
  source 1..21: mol_type = other DNA
cctgcaggtacgtattacaga

SEQ ID NO: 16 - DNA, 34 bp, synthetic construct
  source 1..34: mol_type = other DNA
atacgtacctgcagggcaaggggcgttatgagcc

SEQ ID NO: 17 - DNA, 30 bp, synthetic construct
  source 1..30: mol_type = other DNA
atacgtacctgcaggttgcgggcaaggggc

SEQ ID NO: 18 - DNA, 32 bp, synthetic construct
  source 1..32: mol_type = other DNA
atacgtacctgcagggacgatggggttgcggg

SEQ ID NO: 19 - DNA, 45 bp, synthetic construct
  source 1..45: mol_type = other DNA
atacgtacctgcaggggccattttggaaaaaaatttaataatttt

SEQ ID NO: 20 - DNA, 80 bp, Corynebacterium glutamicum
  source 1..80: mol_type = genomic DNA
gcaaggggcgttatgagccacacttgagtcatcccagtcagacagcaagagtctggcgaacaacagaaagagagatcaca

SEQ ID NO: 21 - DNA, 86 bp, Corynebacterium glutamicum
  source 1..86: mol_type = genomic DNA
ttgcgggcaaggggcgttatgagccacacttgagtcatcccagtcagacagcaagagtctggcgaacaacagaaagagagatcaca

SEQ ID NO: 22 - DNA, 96 bp, Corynebacterium glutamicum
  source 1..96: mol_type = genomic DNA
gacgatggggttgcgggcaaggggcgttatgagccacacttgagtcatcccagtcagacagcaagagtctggcgaacaacagaaagagagatcaca

SEQ ID NO: 23 - DNA, 208 bp, Corynebacterium glutamicum
  source 1..208: mol_type = genomic DNA
ggccattttggaaaaaaatttaataatttttttacgatgaataaaattacattgcccttaaaggtatctaaatgacacttattaaacggtgttcaaaaatggcccagtttttgacgatggggttgcgggcaaggggcgttatgagccacacttgagtcatcccagtcagacagcaagagtctggcgaacaacagaaagagagatcaca

SEQ ID NO: 24 - DNA, 20 bp, synthetic construct
  source 1..20: mol_type = other DNA
ctgtaatacgtacctgcagg

SEQ ID NO: 25 - DNA, 20 bp, synthetic construct
  source 1..20: mol_type = other DNA
ctacgatagccacctgagtg

SEQ ID NO: 26 - DNA, 207 bp, Corynebacterium glutamicum
  source 1..207: mol_type = genomic DNA
ggccattttggaaaaaaatttaataattttttacgatgaataaaattacattgcccttaaaggtatctaaatgacacttattaaacggtgttcaaaaatggcccagtttttgacgatggggttgcgggcaaggggcgttatgagccacacttgagtcatcccagtcagacagcaagagtctggcgaacaacagaaagagagatcaca

SEQ ID NO: 27 - DNA, 207 bp, Corynebacterium glutamicum
  source 1..207: mol_type = genomic DNA
ggccattttggaaaaaatttaataatttttttacgatgaataaaattacattgcccttaaaggtatctaaatgacacttattaaacggtgttcaaaaatggcccagtttttgacgatggggttgcgggcaaggggcgttatgagccacacttgagtcatcccagtcagacagcaagagtctggcgaacaacagaaagagagatcaca

SEQ ID NO: 28 - DNA, 208 bp, Corynebacterium glutamicum
  source 1..208: mol_type = genomic DNA
ggccattttcgaaaaaaatttaataatttttttagggtgaataaaattgcattgcccttaaaggtatctaaatgacccctactgaacggtgttcaaaaatggcccagcttttgacgatggggttgcgggcaaggggcgttatgagccacacttgagtcatcccagtcagacagcaagagtctggcgaacaacagaaagagagatcaca

SEQ ID NO: 29 - DNA, 206 bp, Corynebacterium glutamicum
  source 1..206: mol_type = genomic DNA
ggccattttcgaaaaaaatttaataatttttttacagtgaataaaattgcactgcccttaaaggtatctaaatgacacttattaaacggtgttcaaaaatggcccagttcttgacgatggggttgcggtcgaggggcgttatgggccacacttgagtcatcccagtcaggcagcaagagcctggcgaaaaatagaaagagagacca

SEQ ID NO: 30 - DNA, 206 bp, Corynebacterium glutamicum
  source 1..206: mol_type = genomic DNA
ggccattttcgaaaaaaatttaataatttttttacggtgaataaaattgcactgcccttaaaggtatctaaatgacccttactgaacagtgttcaaaaatggcccagttcttgacgatggggttgcggtcgaggggcgttatgggccacacttgagtcatcccagtcaggcagcaagagcctggcgaacaacagaaaggcagacca

SEQ ID NO: 31 - DNA, 208 bp, Brevibacterium flavum
  source 1..208: mol_type = genomic DNA
ggccattttcgaaaaaaatttaataatttttttagggtgaataaaattgcattgcccttaaaggtatctaaatgacccttactgaacagtgttcaaaaatgattgatttcttggtggcgaggttgcggtcgaggggcgttatgggccacacttgagtcatcccagtcaggcagcaagagcctggcgaacaacagaaagagagatcaca

SEQ ID NO: 32 - DNA, 208 bp, Corynebacterium glutamicum
  source 1..208: mol_type = genomic DNA
ggccattttcgaaaaaaatttaataatttttttagggtgaataaaattgcattgcccttaaaggtatctaaatgatccttattgaacagtgttcaaaaatgattgatttcttggtggcgaggttgcggtcgaggggcgttatgggccacacttgagtcatcccagtcaggcagcaagagcctggcgaacaacagaaagagagatcaca

SEQ ID NO: 33 - DNA, 208 bp, Corynebacterium glutamicum
  source 1..208: mol_type = genomic DNA
ggccattttcgaaaaaaatttaataatttttttacggtgaataaaattgcattgcccttaaaggtatctaaatgacccttactgaacagtgttcaagaatgattgatttcttggtggcgaggttgcggtcgaggggcgttatgagccacacttgagtcatcccagtcaggcagcaagagcctggcgaaaaatagaaagagagaccaca

SEQ ID NO: 34 - DNA, 206 bp, Corynebacterium glutamicum
  source 1..206: mol_type = genomic DNA
ggccattttcgaaaaaaatttaataatttttttacggtgaataaaattgcattgcccttaaaggtatctaaatgacccttactgaacagtgttcaaaaatgattgatttcttggtggcgaggttgcggtcgaggggcattatgggccacacttgagtcatcccagtcaggcagcaagagcctggcgaaaaatagaaagagagacca

SEQ ID NO: 35 - DNA, 208 bp, Corynebacterium glutamicum
  source 1..208: mol_type = genomic DNA
ggcaatttttaaaaaaattttcataaaatttttccgatgaataaaattgcgctgcccttaaaggtatctaaatgacacttattaaacggtgttcaaaaatggcgctgtttttcacgatggggttgcaaccgaccggcgttatgggtcacacttgagtcatcccagtcaggcagcaagagcctggcgaacacaagaaagtgagatcata

SEQ ID NO: 36 - DNA, 206 bp, Corynebacterium glutamicum
  source 1..206: mol_type = genomic DNA
ggccattttcgaaaaaaatttaataatttttttacggtgaataaaattgcactgcccttaaaggtatctaaatgacccttactgaacagtgttcaaaaatgattgatttcttggtggcgaggttgcggtcgaggggcgctatgggccacacttgagtcatcccagtcaggcagcaagagcctggcgaaaaatagaaagagagacca

SEQ ID NO: 37 - DNA, 203 bp, Corynebacterium crudilactis
  source 1..203: mol_type = genomic DNA
attttcgaaaaaaattaataaatttctagggatgaataaaattgcgttgcccttaagggtatctaaatgatccttaatgaacagtgttcaaaaatgactcatttttaaggatcagggttgcatgttggtgacgttataggccaaacttgagtcatcccagtcaggcagcaagagcttggcgaacactagaaagagagatcaca

SEQ ID NO: 38 - DNA, 208 bp, Corynebacterium deserti
  source 1..208: mol_type = genomic DNA
gccttattcgaaaaaaatttagataaattttttacgatgaataaaatagggctgcccttaaaagtatctaaatgacactgactgaacaatgttcaaaaatgcccaattttgtggcgatggggttgcaagtggttgccgggataggccacacttgagtcatcccagtcaggcagcaagagcttggcgaaagaatgaaagtgagatcaca

SEQ ID NO: 39 - DNA, 208 bp, Corynebacterium glutamicum
  source 1..208: mol_type = genomic DNA
ggccattttcgaaaaaaatttaataatttttttaggatgaataaaattgcattgcccttaaaggtatctaaatgacacttattaaacggtgttcaaaaatgattcaaattttggcgacggggttgcggtcgaggggcgttatgggccacacttgagtcatcccagtcagacagcaagagtctggcgaacaacagaaagagagatcaca

SEQ ID NO: 40 - DNA, 208 bp, Corynebacterium glutamicum
  source 1..208: mol_type = genomic DNA
ggccattttcgaaaaaaatttaataatttttttagggtgaataaaattgcattgcccttaaaggtatctaaatgacccctactgaacggtgttcaaaaatggcccagcttttgacgatggagttgcgggcaaggggcgttatgagccacacttgagtcatcccagtcagacagcaagagtctggcgaacaacagaaagagagatcaca

SEQ ID NO: 41 - DNA, 208 bp, Corynebacterium glutamicum
  source 1..208: mol_type = genomic DNA
ggccattttcgaaaaaaatttaataatttttttaggatgaataaaattgcattgcccttaaaggtatctaaatgacacttattaaacggtgttcaaaaatgattcaaattttggcgacggggttgcaatcgataggcgttatgggccacacttgagtcatcccagtcaggcagcaagagcctggcgaacaacagaaagagagatcaca

SEQ ID NO: 42 - protein, 38 aa, Corynebacterium glutamicum; identical to SEQ ID NO: 3

SEQ ID NO: 43 - protein, 38 aa, Corynebacterium glutamicum
MTSVFDIFQSIFDGVHGLVGSIFAGAQGVFDSIVTASS

SEQ ID NO: 44 - protein, 38 aa, Corynebacterium glutamicum
MTSVFDIFQSIFDGVQGLVGSIFAGAQGVFDTIANASS

SEQ ID NO: 45 - protein, 38 aa, Corynebacterium glutamicum
MDSVFAIFQAIFDGVEGLINSVIGGAQGVFDSIKNFSS

SEQ ID NO: 46 - protein, 38 aa, Corynebacterium glutamicum
MESVFDIFQAIFDGVKGLIGSVVGGAQGVFDSIVDFSS

SEQ ID NO: 47 - protein, 38 aa, Brevibacterium flavum
MTSVFEIFQAIFTGVQNLVDSVFAGAQGVFTEVKNASS

SEQ ID NO: 48 - protein, 38 aa, Corynebacterium glutamicum
MTSVFEIFQSIFDGVQALVGSIFAGAQGVFDAVENASS

SEQ ID NO: 49 - protein, 38 aa, Corynebacterium glutamicum
MDSVFDIFQAIFNGVQGLVGSVFNGAQGVFDSIKNFSS

SEQ ID NO: 50 - protein, 38 aa, Corynebacterium glutamicum
MDSVFDIFQAIFDGVKGLVASVFNGAQGVFDSIENFSS

SEQ ID NO: 51 - protein, 38 aa, Corynebacterium glutamicum
MQAIFDIFQSIFDGIQGLVGSVFNGAQGVFDTIQNASS

SEQ ID NO: 52 - protein, 38 aa, Corynebacterium glutamicum
MDSVFAIFQAIFDGVEGLVGSVLGGAQGVFDSIKNFSS

SEQ ID NO: 53 - protein, 38 aa, Corynebacterium crudilactis
MTSVFDIFQSIFDGIQGLVGSVFAGAQGVFDTIVNASS

SEQ ID NO: 54 - protein, 38 aa, Corynebacterium deserti
MTAIFDIFQSIFDGVQGLVGSVFAGAQGVFDSIQNASS

SEQ ID NO: 55 - protein, 38 aa, Corynebacterium glutamicum; identical to SEQ ID NO: 49

SEQ ID NO: 56 - protein, 38 aa, Corynebacterium glutamicum
MTSVFDIFQAIFDGVQGLVGSVFAGAQNVFDSIVTASS

SEQ ID NO: 57 - protein, 38 aa, Corynebacterium glutamicum
MTSVFDIFQSIFDGVQNLVGSIFAGAQGVFDSIVTASS

SEQ ID NO: 58 - DNA, 45 bp, synthetic construct
  source 1..45: mol_type = other DNA
atacgtacctgcaggggccattttcgaaaaaaatttaataatttt

SEQ ID NO: 59 - DNA, 38 bp, synthetic construct; identical to SEQ ID NO: 7
  source 1..38: mol_type = other DNA

SEQ ID NO: 60 - DNA, 17 bp, synthetic construct
  source 1..17: mol_type = other DNA
cgagtggcagtcctacg

SEQ ID NO: 61 - DNA, 45 bp, synthetic construct; identical to SEQ ID NO: 58
  source 1..45: mol_type = other DNA

SEQ ID NO: 62 - DNA, 40 bp, synthetic construct
  source 1..40: mol_type = other DNA
cacctgagtgcgcattttggtctctctttctatttttcgc

SEQ ID NO: 63 - DNA, 45 bp, synthetic construct; identical to SEQ ID NO: 58
  source 1..45: mol_type = other DNA

SEQ ID NO: 64 - DNA, 36 bp, synthetic construct
  source 1..36: mol_type = other DNA
cacctgagtgcgcattttggtctgcctttctgttgt

SEQ ID NO: 65 - DNA, 52 bp, synthetic construct
  source 1..52: mol_type = other DNA
atacgtacctgcaggggccattttcgaaaaaaatttaataatttttttaggg

SEQ ID NO: 66 - DNA, 41 bp, synthetic construct
  source 1..41: mol_type = other DNA
cacctgagtgcgcattgtgatctctctttctgttgttcgcc

SEQ ID NO: 67 - DNA, 45 bp, synthetic construct; identical to SEQ ID NO: 58
  source 1..45: mol_type = other DNA

SEQ ID NO: 68 - DNA, 39 bp, synthetic construct
  source 1..39: mol_type = other DNA
cacctgagtgcgcattgtggtctctctttctatttttcg

SEQ ID NO: 69 - DNA, 45 bp, synthetic construct; identical to SEQ ID NO: 58
  source 1..45: mol_type = other DNA

SEQ ID NO: 70 - DNA, 40 bp, synthetic construct; identical to SEQ ID NO: 62
  source 1..40: mol_type = other DNA

SEQ ID NO: 71 - DNA, 50 bp, synthetic construct
  source 1..50: mol_type = other DNA
atacgtacctgcaggggcaatttttaaaaaaattttcataaaatttttcc

SEQ ID NO: 72 - DNA, 39 bp, synthetic construct
  source 1..39: mol_type = other DNA
cacctgagtgcgcattatgatctcactttcttgtgttcg

SEQ ID NO: 73 - DNA, 51 bp, synthetic construct
  source 1..51: mol_type = other DNA
atacgtacctgcaggtgatgattttcgaaaaaaattaataaatttctaggg

SEQ ID NO: 74 - DNA, 40 bp, synthetic construct
  source 1..40: mol_type = other DNA
cacctgagtgcgcattgtgatctctctttctagtgttcgc

SEQ ID NO: 75 - DNA, 50 bp, synthetic construct
  source 1..50: mol_type = other DNA
atacgtacctgcagggccttattcgaaaaaaatttagataaattttttac

SEQ ID NO: 76 - DNA, 39 bp, synthetic construct
  source 1..39: mol_type = other DNA
cacctgagtgcgcattgtgatctcactttcattctttcg

SEQ ID NO: 77 - DNA, 45 bp, synthetic construct; identical to SEQ ID NO: 58
  source 1..45: mol_type = other DNA

SEQ ID NO: 78 - DNA, 38 bp, synthetic construct; identical to SEQ ID NO: 7
  source 1..38: mol_type = other DNA

SEQ ID NO: 79 - DNA, 46 bp, synthetic construct
  source 1..46: mol_type = other DNA
atacgtacctgcaggggccattttcgaaaaaaatttaataattttt

SEQ ID NO: 80 - DNA, 38 bp, synthetic construct; identical to SEQ ID NO: 7
  source 1..38: mol_type = other DNA

SEQ ID NO: 81 - DNA, 45 bp, synthetic construct; identical to SEQ ID NO: 58
  source 1..45: mol_type = other DNA

SEQ ID NO: 82 - DNA, 38 bp, synthetic construct; identical to SEQ ID NO: 7
  source 1..38: mol_type = other DNA

SEQ ID NO: 83 - DNA, 32 bp, synthetic construct
  source 1..32: mol_type = other DNA
ataaaattacattgcccttaaaggtatctaaa

SEQ ID NO: 84 - DNA, 45 bp, synthetic construct
  source 1..45: mol_type = other DNA
gcaatgtaattttattcatcgtaaaaaattattaaatttttttcc

SEQ ID NO: 85 - DNA, 35 bp, synthetic construct
  source 1..35: mol_type = other DNA
aataatttttttacgatgaataaaattacattgcc

SEQ ID NO: 86 - DNA, 35 bp, synthetic construct
  source 1..35: mol_type = other DNA
cgtaaaaaaattattaaattttttccaaaatggcc

SEQ ID NO: 87 - DNA, 27 bp, synthetic construct
  source 1..27: mol_type = other DNA
ctaaatgatccttattgaacagtgttc

SEQ ID NO: 88 - DNA, 29 bp, synthetic construct
  source 1..29: mol_type = other DNA
ataaggatcatttagatacctttaagggc

SEQ ID NO: 89 - DNA, 25 bp, synthetic construct
  source 1..25: mol_type = other DNA
gctatgggccacacttgagtcatcc

SEQ ID NO: 90 - DNA, 31 bp, synthetic construct
  source 1..31: mol_type = other DNA
agtgtggcccatagcgcccctcgaccgcaac

SEQ ID NO: 91 - DNA, 206 bp, synthetic construct
  source 1..206: mol_type = other DNA; note = PcgYImut
ggccattttcgaaaaaaatttaataatttttttacggtgaataaaattgcattgcccttaaaggtatctaaatgacccttactgaacagtgttcaaaaatgattgatttcttggtggcgaggttgcggtcgaggggcgctatgggccacacttgagtcatcccagtcaggcagcaagagcctggcgaaaaatagaaagagagacca

SEQ ID NO: 92 - DNA, 26 bp, synthetic construct
  source 1..26: mol_type = other DNA
gcactgcccttaaaggtatctaaatg

SEQ ID NO: 93 - DNA, 25 bp, synthetic construct
  source 1..25: mol_type = other DNA
ctttaagggcagtgcaattttattc

SEQ ID NO: 94 - DNA, 1000 bp, Corynebacterium glutamicum
  source 1..1000: mol_type = genomic DNA
ccaacttggtagtcctgggtatacagattctcgccatgcaagaatgcattagcaccggcgcggtacacgtcagtatcaatatggaagaagaaaacaaaagactcgatggcccgaacattgaaaattgaaggccataaagtcaagagtagagcgatggtagaaagcactaacagtgcttttctcagcgtctgatttgtagccatatcgcgccattggaattgactgagatttccctcagtgccatccacaagtttttcaccgtgcatgaaaaatagtgtatccgtatccagcggtttttaaggaactgagctgtgcaccttgtgaccttttgtgacactgctcaatgctttacggctacgatgaacaacaaaccgacgttttcgacgctgtgaaggactaattgctagtgcgttatttttacgatactgagttcattgaagatgggcgcacgatcgaattggtctctattggaatcgtcgcagaagacggtcgcgagtattacgcagttagcacacagtttgattcctccaaggcgaacgcttgggtgcgcgccaacgtgttggacaaattgcctaatccttcctccaaagtgtggaaatctgcagacactataaagcgcgaagtttatgagtttctcacctccaccggaccaacccctgaactgtgggcctgggtgggcgcatatgaccacgtgttgttggcacaaatgtggggcgatatggcggggcttcctcgggagatccctcgttttacccgcgagcttcgccagtattgggacatggctggccgcccaacgctgccagagctgccgaacggcaaccacgatgcgttgattgatgcgcgtcataatttagccaagttcaaagtgtgcatggcagcgctgcctttgggtaaaagggatcgcgtctcttagtcgatctgctcccattccataggttgggagaaaacttaactgttattccattccttaaaacaccgatatcgtgctatgaataggggt

SEQ ID NO: 95 - DNA, 35 bp, synthetic construct
  source 1..35: mol_type = other DNA
aaaacgacggccagtccaacttggtagtcctgggt

SEQ ID NO: 96 - DNA, 35 bp, synthetic construct
  source 1..35: mol_type = other DNA
ggatctaaacgatctacccctattcatagcacgat

SEQ ID NO: 97 - DNA, 1000 bp, Corynebacterium glutamicum
  source 1..1000: mol_type = genomic DNA
gtgagttggacagttgatatccctaaagaagttctccctgatttgccaccattgccagaaggcatgcagcagcagttcgaggacaccatttcccgtgacgctaagcagcaacctacgtgggatcgtgcacaggcagaaaacgtgcgcaagatccttgagtcggttcctccaatcgttgttgcccctgaggtacttgagctgaagcagaagcttgctgatgttgccaacggtaaggccttcctcttgcagggtggtgactgtgcggaaactttcgagtcaaacactgagccgcacattcgcgccaacgtaaagactctgctgcagatggcagttgttttgacctacggtgcatccactcctgtgatcaagatggctcgtattgctggtcagtacgcaaagcctcgctcttctgatctggatggaaatggtctgccaaactaccgtggcgatatcgtcaacggtgtggaggcaaccccagaggctcgtcgccacgatcctgcccgcatgatccgtgcttacgctaacgcttctgctgcgatgaacttggtgcgcgcgctcaccagctctggcaccgctgatctttaccgtctcagcgagtggaaccgcgagttcgttgcgaactccccagctggtgcacgctacgaggctcttgctcgtgagatcgactccggtctgcgcttcatggaagcatgtggcgtgtccgatgagtccctgcgtgctgcagatatctactgctcccacgaggctttgctggtggattacgagcgttccatgctgcgtcttgcaaccgatgaggaaggcaacgaggaactttacgatctttcagctcaccagctgtggatcggcgagcgcacccgtggcatggatgatttccatgtgaacttcgcatccatgatctctaacccaatcggcatcaagattggtcctggtatcacccctgaagaggctgttgcatacgctgacaagctcgatccgaacttcgagcctggccgtttgacca

SEQ ID NO: 98 - DNA, 35 bp, synthetic construct
  source 1..35: mol_type = other DNA
ccaggaggacatacagtgagttggacagttgatat

SEQ ID NO: 99 - DNA, 35 bp, synthetic construct
  source 1..35: mol_type = other DNA
atcctctagagtcgatggtcaaacggccaggctcg

SEQ ID NO: 100 - DNA, 362 bp, synthetic construct
  source 1..362: mol_type = other DNA; note = DNA fragment containing tu promoter
agatcgtttagatccgaaggaaaacgtcgaaaagcaatttgcttttcgacgccccaccccgcgcgttttagcgtgtcagtaggcgcgtagggtaagtggggtagcggcttgttagatatcttgaaatcggctttcaacagcattgatttcgatgtatttagctggccgttaccctgcgaatgtccacagggtagctggtagtttgaaaatcaacgccgttgcccttaggattcagtaactggcacattttgtaatgcgctagatctgtgtgctcagtcttccaggctgcttatcacagtgaaagcaaaaccaattcgtggctgcgaaagtcgtagccaccacgaagtccaggaggacataca

SEQ ID NO: 101 - DNA, 20 bp, synthetic construct
  source 1..20: mol_type = other DNA
agatcgtttagatccgaagg

SEQ ID NO: 102 - DNA, 20 bp, synthetic construct
  source 1..20: mol_type = other DNA
tgtatgtcctcctggacttc

SEQ ID NO: 103 - DNA, 20 bp, synthetic construct
  source 1..20: mol_type = other DNA
tcgactctagaggatctact

SEQ ID NO: 104 - DNA, 20 bp, synthetic construct
  source 1..20: mol_type = other DNA
actggccgtcgttttacaac

SEQ ID NO: 105 - DNA, 20 bp, synthetic construct
  source 1..20: mol_type = other DNA
cgctacaactggcgcatcga

SEQ ID NO: 106 - DNA, 20 bp, synthetic construct
  source 1..20: mol_type = other DNA
gtcgttgagtgtttcagtcc

SEQ ID NO: 107 - DNA, 1000 bp, Corynebacterium glutamicum
  source 1..1000: mol_type = genomic DNA
atccctgaaggttcctccatatcagagctcggcccagagttggaagaacgagatatcgtggccaccaactcagcgttccaaacagcggccagcaacaaccccaacgcgggtagtgtacagccaggtttctaccgtctgcaggaacaaatgaacgcagcagctgcagtgtcggctctgcttgatccagacaaccaggttgatctcctcgacattcacggcggcgccaccttgatggacgtcactgttgtcggcggaaacacccgcgcgggaatctactcccagatcgcagccgtgacctgcaccgaaggctccgccaactgcatcaccgctgaggatttgcagcaggttgcctccaccgtgtcgcctgcagaattgggtgtcccagattgggcaatcgctgctgtggaagctcgcggaactgatccaaagcgcctcgaaggcctgatcatgcctggccaatacgtggtggatccatccaacgacgcccagggaatcctcaccgatctgatcacgcgatcagcaaaccatttccaagaaaccgacatcacgggccgtgcagatgccatcggacttactccatatgagctgctcaccgcagcatctctaatcgagcgcgaagcaccagcaggagattttgataaggtcgcccgcgtcatcttgaaccgtctcgccgagccaatgcagctgcaattcgactccaccgtcaactacggtctgtctgaacaagaagtagcaaccaccgacgaagaccgtcagaccgtcaccccatggaacacttacgccatggacggcctgccacaaacccccatcgccgcagtatccaccgaagcactccaagccatggaaaaccctgcagaaggaaactggctgtactttgtcaccatcgacaccgatggaaccaccgtgttcaacgacaccttcgaagagcacgaagccgacattgagcaagctttgaacagtggcgttctagacagcaaccgataaggatcagcgaataaaa

SEQ ID NO: 108 - DNA, 35 bp, synthetic construct
  source 1..35: mol_type = other DNA
aaaacgacggccagtatccctgaaggttcctccat

SEQ ID NO: 109 - DNA, 35 bp, synthetic construct
  source 1..35: mol_type = other DNA
ggatctaaacgatctttttattcgctgatccttat

SEQ ID NO: 110 - DNA, 1000 bp, Corynebacterium glutamicum
  source 1..1000: mol_type = genomic DNA
atgggttctcacatcactcaccgggcggccgtactcggctcacccatcgagcattccaaatccccagtcctccacaacaccggctataaagccctcggactggaccaatgggaatacgaccgctttgagtgcaccggcgacatgctccccggcatcgtctccggcgctgatgaaacctactgcggattctccgtcaccatgccgtctaaattcgcagctcttgaattcgccgacgaagtaaccgaacgcgcctgcgccatcggctccgcaaacaccttgctgcgcacggccaccggatggcgcgccgacaacaccgacgtcgacggcatcaggggagctctcggtgaactcctcggcggcgcatcactggccggcaaacacgccatcgtcatcggctccggcggcaccgcacgccccgccatctgggcactcatcgaagccggggtcgcccggatcacggtgctcaaccgctccgatcgcaccgccgaactgcaaacgcttttcgacgaaacccccaccaccttggcctacgccccgctcgagcatctccacatcgaagccgacgtcgtagtctctacagtgccctccgcagcaatcgcaggcctcgaagacacccttgcgatcgccccagtcctcgacgtcatctacgacccctggccaacaccactcgtagaagtcacacgagccaaaggcctcaaagctgtcggaggccacgtcatgctggcacaccagtcctacggacagtttgaacaattcaccggaatggatgcaccccgcgatgccatgcgtgaggctttggaagagtctttaggcatctcagaagaacactaagtccccgccacctcctcaacaaaactcctagtgacgcttgaaccgaaggtggacttcatcgcctaggtcaaagcgctcaacacgaacgccatacacaggttccaaatgctctggggtcaatacctctgagggcgttccttgagtaaccacacgtccttggtcaaggagg

SEQ ID NO: 111 - DNA, 35 bp, synthetic construct
  source 1..35: mol_type = other DNA
ccaggaggacatacaatgggttctcacatcactca

SEQ ID NO: 112 - DNA, 35 bp, synthetic construct
  source 1..35: mol_type = other DNA
atcctctagagtcgacctccttgaccaaggacgtg

SEQ ID NO: 113 - DNA, 20 bp, synthetic construct
  source 1..20: mol_type = other DNA
cgacctcaacctcgcagctg

SEQ ID NO: 114 - DNA, 20 bp, synthetic construct
  source 1..20: mol_type = other DNA
gtagccacctcaaaccggac

SEQ ID NO: 115 - DNA, 1000 bp, Corynebacterium glutamicum
  source 1..1000: mol_type = genomic DNA
gttcctggatgacaacggcgtataccgcaacaccaaccgtgcaggtggcctcgaaggcggcatgaccaacggtgaaaccctgcgcgttcgtgctggcatgaagccaatttctactgtgcctcgcgccctgaaaaccattgatatggaaaacggcaaggcagcaaccggaatccaccagcgttccgacgtgtgcgctgttccagccgccggtgtcgttgcagaagcaatggtcaccctggttctcgcccgcgcagtcctgcagaaattcggcggtgactccctgagcgaaaccaagagcaacattgacacctacctcaaaaacattgaggaacgaatgaaattcgaaggtttagaggatggagcgtaatgaagtgaatgatcaaattcacttagatcatcaatcagatgacacctctgaatgctcctgcccgatcgtggttcttgtgggtttgccaggagctggaaaatccaccattggacgtcgattagcgcgcgccttaaacactgaactcgtcgactccgacgaactgattgagcgcgccaccggaaaagcctgtggcgccgtgttcagcgagctcggcgagccagccttccgcgagctcgaggccatccacgtggccgaagcactgaaatcctccggagtggtgagcttgggaggcggatctgtgctgacagaatccacccgtgaactgctcaaaggccaggacgtggtctggatcgacgtgccagtagaagaaggcatcaggcgcaccgcaaacgagcgttcccgccccgtgctgcaagccgccgaccccgccgagcactaccgcaacctggtgaaagtgcgcaccccgttgtacgaagaggtggcaacctaccgacttcgcaccaacaaccgcagcccccagcaagtggtggcagcagtgttgcatcatctagaaatcgattaattaaaccgggcacctgattaacattgggctgcccggtttcttcctattacaagcgaaaggcaacgtgcccc

SEQ ID NO: 116 - DNA, 35 bp, synthetic construct
  source 1..35: mol_type = other DNA
aaaacgacggccagtgttcctggatgacaacggcg

SEQ ID NO: 117 - DNA, 35 bp, synthetic construct
  source 1..35: mol_type = other DNA
ggatctaaacgatctggggcacgttgcctttcgct

SEQ ID NO: 118 - DNA, 1000 bp, Corynebacterium glutamicum
  source 1..1000: mol_type = genomic DNA
atgagcgcagtgcagattttcaacaccgtccacgtcaatggatcttccccctatgatgtccacattggttccggcctcaacgagctcattgttcagcgcgcagcggaatcaggcgcggagcaggtagcgattttgcaccagcccagcatggatgacattgcatccgagttggatgcagcactagtcgctgctggtttgaaggtcctgcaccttaatgttcccgatgcggaaaacggcaagtccttggaagtagcggggcagtgctgggatgaattgggtggcgcagcattcggccgccgcgatatcgtcatcggacttggtggcggtgctgccacagatctcgcgggattcgtcgctgctgcatggatgcgtggcgtgcgcgtcattcaggttccaaccaccttgttggccatggtggacgctgcggtgggcggcaagactggcatcaataccgccgcaggcaagaaccttgtgggcgcgttccacgagcctgacgcagtattcattgacaccgatcgcctagccaccctgcctgacgcggaaatcatcgcgggatccgccgaaatcatcaaaactggtttcatcgccgacccagaaatcctgcgcctttacgaaactgatcccgcagcctgcctgaagaaagaagtcgaaggctcccacctacctgaactgatttggcgctccgtcaccgtcaagggctccgtggtcggccaagacctcaaagaatctagcctgcgcgaaatcctcaactacggacacacctttgcccacgccgtcgaactccgcgaaaacttccgctggcgccacggcaatgccgttgcagtgggcatgatgttcatcgccaacctctcccacaagctcgggcttatcgacgcgcccctcctcgagcgccaccgctcaatcctggcggccatcggtctgcccacttcctacgaaggcggagccttcgacgagctttacgacggtatgacccgcgacaagaaaaaccgcgacggcaaca

SEQ ID NO: 119 - DNA, 35 bp, synthetic construct
  source 1..35: mol_type = other DNA
ccaggaggacatacaatgagcgcagtgcagatttt

SEQ ID NO: 120 - DNA, 35 bp, synthetic construct
  source 1..35: mol_type = other DNA
atcctctagagtcgatgttgccgtcgcggtttttc

SEQ ID NO: 121 - DNA, 20 bp, synthetic construct
  source 1..20: mol_type = other DNA
ctcctgctgcgagtaaatct

SEQ ID NO: 122 - DNA, 20 bp, synthetic construct
  source 1..20: mol_type = other DNA
caggagctggaaaatccacc

SEQ ID NO: 123 - DNA, 1000 bp, Corynebacterium glutamicum
  source 1..1000: mol_type = genomic DNA
caccaccgcctacgctccaacccgagaaatgcgcgtctacatcaaaggtctacgcaccacctgtagcgtccctggctgcagtgtagcggtcgaaaactgccaactggaccacatcatcccctggggtgaaggagggccgacaacaccgtggaatattcatcccctgtgtgtcttccaccacatccagaagactgaagggaggctccagtgctatccactaccggacggcaccgtcctattcctagtggatggaataccggtgttctccatccccgacgggcctttatctaaatcgaataaaacctgggggacaaagttcggcaaatacatggagcgtcgaatcgccgcctaatccagcaagccagcgtgatcgttacgcacgttccccacatcagacgacacctctcggacactcaagcgcttcacccactcttgagaaaccggatgcaacatctctttagcttcctcagctgtaccaaacagccattgctccaactcgtcatgctccaaaaaccgtggcaaacgattatgcaaccatgcaatcggctccacagattcggtcgtcaccatcgtcgccgacatctgatctaaaccagtcgaccacaaacccgcagcccacatcagctcatcacctaaagaaacaaaatgaggcttcttatcgtgccattcgtaataaccatccatcggaattaaacaacgctgctgtttaaatgcatcacgaaacgacggcttctccgccaccgtctcgccacgtgcattaaaaagcggaggacctgaatcatccttcttccaatgcggaaacaatccccaacgcgccggttccaaaagcatctcttccccggggcgaacgatcggaattatctgagtcggagcaaggttgtatcgcggtcccggagttccttgcggagccacgactgatcggtcaagtgctatctcggttgcatcaataagcgaatcaccggtggtgaacaaaacaaatcttccacacataacatctatt

SEQ ID NO: 124 - DNA, 35 bp, synthetic construct
  source 1..35: mol_type = other DNA
aaaacgacggccagtcaccaccgcctacgctccaa

SEQ ID NO: 125 - DNA, 35 bp, synthetic construct
  source 1..35: mol_type = other DNA
ggatctaaacgatctaatagatgttatgtgtggaa

SEQ ID NO: 126 - DNA, 1000 bp, Corynebacterium glutamicum
  source 1..1000: mol_type = genomic DNA
atggtctttgtgtctgattcgtctatctctttgcccatttgggatgctccgcgcgctcgcggccccatagtctcggacctggctatccctggttccaagtcgatcaccaaccgcgccctcatcttggctgcgctcgcatcaactccatccaccatcattgatgtccttcgtagtcgtgataccgatctcatgactgatggtctacgcagcctcggaatcaccattactgaagaggcagtcgatcgctaccgcgttgagcccggacagttgtctgctggctccgttgagtgtggtcttgctggtacggtcatgcgctttttgcctcctgttgctgctttcgctgatggtcctgttcattttgatggcgatcctcaagctcgtgttcgtccgatgaccagcattttggatgcgctgcgttcgcttggtgtggaggtagacaacaacaatctgcctttcactgttaatgctggtgaggtccctgagggtggcgtggttgagattgatgcttccggctcatctcagtttgtttctggtcttttgctttcagcgcctcgttttaaaaatggcgtcaccgttaagcacgtcggtggtcgtctgccgagcatgccgcatattgagatgaccgtcgatatgcttcgttccgcaggcattgagatcgaagagtcagaaaatcagtgggttgttcatcctggtgagatcttgggtcggacctggcgcattgagccggatctttctaatgcgactccgttcctagctgccgctgcggtcactggtggaaccatcaagattaaccactggccaatcaaaactactcagcctggcgatgctattcgttcgattcttgagcgcatgggctgcgaagttgagctggttgctcagggtgaaggttacgatctgtcggtgactggtccggttgctctcaagggcattgagatcgatatgtccgatatcggtgagttgacccctaccgtggcggcgttggctgcgttggcgtcgacag

SEQ ID NO: 127 - DNA, 35 bp, synthetic construct
  source 1..35: mol_type = other DNA
ccaggaggacatacaatggtctttgtgtctgattc

SEQ ID NO: 128 - DNA, 35 bp, synthetic construct
  source 1..35: mol_type = other DNA
atcctctagagtcgactgtcgacgccaacgcagcc

SEQ ID NO: 129 - DNA, 20 bp, synthetic construct
  source 1..20: mol_type = other DNA
cgcagccaaacgatccgtct

SEQ ID NO: 130 - DNA, 20 bp, synthetic construct
  source 1..20: mol_type = other DNA
cgaaccacgtccagtcggga

SEQ ID NO: 131 - DNA, 1000 bp, Corynebacterium glutamicum
  source 1..1000: mol_type = genomic DNA
gtggtcatttatacctcgcggccagcggcgaaacgatcaagtgcaccagtcctcgccaacgcgcggaccaggtaccagctgagcaggccggcaaggatcgcaccggaaataaggacagtggtggaatagatgatgttgaaggacatcgtctttgcgaggtttccgtagaagaacatttccaggaaaattgcgccgccacctgcgcccatacctgcaagcatggtggtgggcaggctgtagcgacggtagaggaacagcgcgaagatgatttcagcgccgattccctgcgccaagccggagtaaatggtggagataccaaactgtgaagcaagcgctgcagagacacatgcggccactacttcaacgaaaattgcggcacccggcttgcggataaccaacccaccgagcacaccaccgagcagccaaataccaatggcgatgccgccaaggcctggtgtgagtgcgtgaaatgcggtggtccaggcgtagccgatggaattccacacgatgaaaatcaatccgcaggcgacacccaaaacggatgcgatgacgatgtcaataacacgccaggaagactttggttgattagttttttgcatggcaggactagccatatttttcctccctatcgccggcattatccggatcaggttcgacggtcgtggctatgccagatctcagcccggattttcaccgagcacccgtgtctatgaaatttaagtacgcgttcacagtagcttaaaccaattggaaatcctagaaactgacctagattaatacataaccaccccaacccctgacacacacccctaattacaccctggcagcatgagctgaaacgcttttccgctggctgtgacttcaacctcagaaaatgcctggttcgcaaggcgaacaggttgtcacggaatgcactttcacttacattgagtcccaaatcactgtgaggtgcaccatttaatggacttcacctccagtgggtcaatgaaaggagttcccc

SEQ ID NO: 132 - DNA, 35 bp, synthetic construct
  source 1..35: mol_type = other DNA
aaaacgacggccagtgtggtcatttatacctcgcg

SEQ ID NO: 133 - DNA, 35 bp, synthetic construct
  source 1..35: mol_type = other DNA
ggatctaaacgatctggggaactcctttcattgac

SEQ ID NO: 134 - DNA, 1000 bp, Corynebacterium glutamicum
  source 1..1000: mol_type = genomic DNA
acgctcgtgtcaacgaccaccccaacccgcgcaaccaaaagtgtcggaacagttctcgcactcctgtggttcgcaattgtcctcgacggctttgacctagtcgtcctgggtgcaacaatcccgtccatgctggaggatcccgcgtgggatctcactgctggacaggccacacagatttccaccatcggcctcgtcggcatgaccattggcgcactgaccatcggtttcttaacggaccgtctgggtcgacgccgtgtcatgctgttctctgtggcagtattttctgtattcactctcctgctggcattcaccaccaacgtccagctcttcagcctgtggcgtttcctcgcaggtgttggccttggtggagcactccccaccgcaattgccatggtgaccgagttccgccccggcaccaaagcgggctctgcatccaccaccttgatgaccggctaccacgtcggcgcagtagcaaccgccttccttggcctcttccttatcgacggctttggttggcactccatgttcatcgcaggtgccgtaccaggactgatcctgctaccactgctgtacttcttccttccagaatccccgcagtacctcaaaatctccggcaagttggatgaggcgcaggcagttgcagcatcttatggactttccctggatgatgatcttgatcgcgaacacgaagaagaactcggcgagtcctcctcactttcctccctgttcaagccctcgttccgccgcaacaccctggcgatttggggcacctcattcatgggactcctcctggtctacggcctgaacacatggctgccacaaatcatgcgccaagcagactacgacatgggtaactcgcttggattcctcatggtgctcaacatcggcgcagtgatcggcctttatattgcagggcgaattgccgataagaactcccctcgcaaaacagcactcgtatggttcgtgttctctgcattttccctcgcgttgcttgctgtcc

SEQ ID NO: 135 - DNA, 35 bp, synthetic construct
  source 1..35: mol_type = other DNA
aatctcaaaaagtagacgctcgtgtcaacgaccac

SEQ ID NO: 136 - DNA, 35 bp, synthetic construct
  source 1..35: mol_type = other DNA
atcctctagagtcgaggacagcaagcaacgcgagg

SEQ ID NO: 137 - DNA, 438 bp, Corynebacterium glutamicum
  source 1..438: mol_type = genomic DNA
atgcctggaaaaattctcctcctcaacggcccaaacctgaacatgctgggcaaacgcgagcctgacatttacggacacgacaccttggaagacgtcgtcgcgctggcaaccgctgaggctgcgaagcacggccttgaggttgaggcgctgcagagcaatcacgaaggtgagctaatcgatgcgctgcacaacgctcgcggcacccacatcggttgcgtgattaaccccggcggcctgactcacacttcggtggcgcttttggatgctgtgaaggcgtctgagcttcctaccgttgaggtgcacatttccaatccgcatgcccgtgaagagttccgccaccattcttacatttccctcgccgcggtctccgttatcgctggcgctggcatccagggttaccgtttcgcggtcgatatcctggcaaatctcaaaaagtag

SEQ ID NO: 138 - DNA, 35 bp, synthetic construct
  source 1..35: mol_type = other DNA
ccaggaggacatacaatgcctggaaaaattctcct

SEQ ID NO: 139 - DNA, 20 bp, synthetic construct
  source 1..20: mol_type = other DNA
ctactttttgagatttgcca

SEQ ID NO: 140 - DNA, 20 bp, synthetic construct
  source 1..20: mol_type = other DNA
gtacctgggagctgaacaca

SEQ ID NO: 141 - DNA, 20 bp, synthetic construct
  source 1..20: mol_type = other DNA
gaagttgatgtctttgagcg

SEQ ID NO: 142 - DNA, 1037 bp, Corynebacterium glutamicum
  source 1..1037: mol_type = genomic DNA
gtctagacccggcaattgaacccatgccgaaaaatgaattcttcaatctatatgggggtatgtggaaaacctaaaatcaagaggactcccagcacatgcgataaaatctcacatgtcgtttgatactgcaaagtaccgaatcgcactgttagtttttcaagggaagccggttaacaatccggcgctgacccgcaaccgtagatcaccttcgcctggagttttcacgcaaaggggacaagccggattacttggaaaactgacattgacttagaacctttttgtcgtggactacgaaaagcttgcatcttcaaattctgcgcacaaagtgttctaagacgacgtctgcccatcggcgctctaatgcacattacagcgtttacagaattgaaaatgaaaggttcaaagccttgaccattacttttagccgcgttgctctgaccaccctggcagtcaccgcaaccactttgtccctgagcactgctgcgaatgcacagtcttccttgttggataagactcttgatgcccgtcagtgcatcgatgcagacaacgtctgggtctcagttgactatggtgcagattccgaaaaagaaccagagggcgcatgtgccaccgagttcactgatggtgttgtagctcttgaatctgctgggttcaaactgacctttgacgaatctgaaatgggcaaatacatgaccggtatcaacggagttgttcctgattgggttgaaactggaacttactggagttactactctggtgaagtcgcagatgattacagcgtggactacacctactacgaggttggtgcatctaattctgaacctgaaggtggaactgttgaggcttgggttgttggcaccggcgaggaaacaccagcactcgagactcttcctgaaactccagcagcaaccggatcttctgaagacggcggctggattgcagtcatcgcaggtcttctcgcactgatcggtggtggagttgcagctttgtaccagggcttgatcactatcccaggtctggttctgcctaagttttaa

SEQ ID NO: 143 - DNA, 35 bp, synthetic construct
  source 1..35: mol_type = other DNA
aaaacgacggccagtgtctagacccggcaattgaa

SEQ ID NO: 144 - DNA, 35 bp, synthetic construct
  source 1..35: mol_type = other DNA
ctggcccagctggccttaaaacttaggcagaacca

SEQ ID NO: 145 - DNA, 994 bp, Corynebacterium glutamicum
  source 1..994: mol_type = genomic DNA
caacctaacctaaagcttcaaacaagagtgcccaccgacccttcaagatcggtgggcactttaggtttgctccacgaagcaagccaacaaaatctttagacccgaggcaccccggcctccccgaagtcacgctcgacgccgaaagcggcgcggcggctggcgcgtcgtaaagcacctaaaacgggtttggctgtgagcagtaatagcactgaggtgaagaaggcgcggccgagatcccaacccatggatgtggtgaggcagaacagcatgaaggtgtggaggttttccaggacgggcgcgccgggtgtgaaggaaagcccgctggtgacaccgatggcgtagggccagaagctcatgttcatcatggttccgtagccgagtgaagagacgatggcgtataggacgatgatgagcatttcctttttgccgcgtacttgggggagtaggccggcgccgaagctgacccaggcggctgcgagcatttggtaggggagccacggtccgattcctgcggtgagcagcgcggatgcgaacagtccggtgttgccgaggatgaatccgaagccgggtccgaaggctcgtccgccgaggatgaggacaaagaagactgcttcaaagcctgctgcgccggcaccgaatggtcggactacggcaaccatggcggtgaggacgccgagcatggctacggctttaacgtcgaatccgttttcactgatttcggcgatgacagcggccagcacgaggggaatgacgatcgcgatgtagaggggcgcttgggctttgtcggacaggaaggattccgggttgacgatcagcggccagaagaaaatcacgatgctcaaaaccgcaaggaagcttaaggtgaggaaggttttgggcttgagtgtgatggcgttgatcatgagatttcaccatgccctagcgcagctttcacggccgagactgtgagccagtgtgattcctcttggatgccggcggtgatttttgcgacttg

SEQ ID NO: 146 - DNA, 35 bp, synthetic construct
  source 1..35: mol_type = other DNA
aggcccacgtggccgcaacctaacctaaagcttca

SEQ ID NO: 147 - DNA, 35 bp, synthetic construct
  source 1..35: mol_type = other DNA
tcctctagagtcgaccaagtcgcaaaaatcaccgc

SEQ ID NO: 148 - DNA, 377 bp, synthetic construct
  source 1..377: mol_type = other DNA; note = DNA fragment containing tu promoter
ggccagctgggccagatcgtttagatccgaaggaaaacgtcgaaaagcaatttgcttttcgacgccccaccccgcgcgttttagcgtgtcagtaggcgcgtagggtaagtggggtagcggcttgttagatatcttgaaatcggctttcaacagcattgatttcgatgtatttagctggccgttaccctgcgaatgtccacagggtagctggtagtttgaaaatcaacgccgttgcccttaggattcagtaactggcacattttgtaatgcgctagatctgtgtgctcagtcttccaggctgcttatcacagtgaaagcaaaaccaattcgtggctgcgaaagtcgtagccaccacgaagtccaggaggattaattaa

SEQ ID NO: 149 - DNA, 20 bp, synthetic construct
  source 1..20: mol_type = other DNA
ggccagctgggccagatcgt

SEQ ID NO: 150 - DNA, 20 bp, synthetic construct
  source 1..20: mol_type = other DNA
ttaattaatcctcctggact

SEQ ID NO: 151 - DNA, 35 bp, synthetic construct
  source 1..35: mol_type = other DNA
aggaggattaattaaatgaattatcagaacgacga

SEQ ID NO: 152 - DNA, 20 bp, synthetic construct
  source 1..20: mol_type = other DNA
ttacccgcgacgcgctttta

SEQ ID NO: 153 - DNA, 1176 bp, synthetic construct
  source 1..1176: mol_type = other DNA; note = DNA fragment containing mutant aroG gene
atgaattatcagaacgacgatttacgcatcaaagaaatcaaagagttacttcctcctgtcgcattgctggaaaaattccccgctactgaaaatgccgcgaatacggttgcccatgcccgaaaagcgatccataagatcctgaaaggtaatgatgatcgcctgttggttgtgattggcccatgctcaattcatgatcctgtcgcggcaaaagagtatgccactcgcttgctggcgctgcgtgaagagctgaaagatgagctggaaatcgtaatgcgcgtctattttgaaaagccgcgtaccacggtgggctggaaagggctgattaacgatccgcatatggataatagcttccagatcaacgacggtctgcgtatagcccgtaaattgctgcttgatattaacgacagcggtctgccagcggcaggtgagtttttaaatatgatcaccccacaatatctcgctgacctgatgagctggggcgcaattggcgcacgtaccaccgaatcgcaggtgcaccgcgaactggcatcagggctttcttgtccggtcggcttcaaaaatggcaccgacggtacgattaaagtggctatcgatgccattaatgccgccggtgcgccgcactgcttcctgtccgtaacgaaatgggggcattcggcgattgtgaataccagcggtaacggcgattgccatatcattctgcgcggcggtaaagagcctaactacagcgcgaagcacgttgctgaagtgaaagaagggctgaacaaagcaggcctgccagcacaggtgatgatcgatttcagccatgctaactcgtccaaacaattcaaaaagcagatggatgtttgtgctgacgtttgccagcagattgccggtggcgaaaaggccattattggcgtgatggtggaaagccatctggtggaaggcaatcagagcctcgagagcggggagccgctggcctacggtaagagcatcaccgatgcctgcatcggctgggaagataccgatgctctgttacgtcaactggcgaatgcagtaaaagcgcgtcgcgggtaagcggccgcttgccctgctgtttttagcttcaacccggggcaatatgattctccggaattttattgccccgggttgttgttgttaatcggtacaaagggtcttaagcacaggcccacgtggccg

SEQ ID NO: 154 - DNA, 20 bp, synthetic construct
  source 1..20: mol_type = other DNA
gccgtgaaagctgcgctagg

SEQ ID NO: 155 - DNA, 20 bp, synthetic construct
  source 1..20: mol_type = other DNA
gcacattacagcgtttacag

SEQ ID NO: 156 - DNA, 18 bp, synthetic construct
  source 1..18: mol_type = other DNA
atggtgagcaagggcgag

SEQ ID NO: 157 - DNA, 20 bp, synthetic construct
  source 1..20: mol_type = other DNA
ctacttgtacagctcgtcca

SEQ ID NO: 158 - DNA, 22 bp, synthetic construct
  source 1..22: mol_type = other DNA
ctatgccaagcttctttcaccc

SEQ ID NO: 159 - DNA, 35 bp, synthetic construct
  source 1..35: mol_type = other DNA
gagctgtacaagtagggaggtttaaacaagcggcc

SEQ ID NO: 160 - DNA, 35 bp, synthetic construct
  source 1..35: mol_type = other DNA
agaagcttggcatagctcaacatgcgcgaaaatgg

SEQ ID NO: 161 - DNA, 39 bp, synthetic construct
  source 1..39: mol_type = other DNA
gcccttgctcaccattgtgatctctctttctgttgttcg

SEQ ID NO: 162 - DNA, 18 bp, synthetic construct
  source 1..18: mol_type = other DNA
tgtaaaacgacggccagt

SEQ ID NO: 163 - DNA, 20 bp, synthetic construct
  source 1..20: mol_type = other DNA
ggccttttgctcacatgttc

SEQ ID NO: 164 - DNA, 34 bp, synthetic construct
  source 1..34: mol_type = other DNA
agaagcttggcatagtagcgtgtcagtaggcgcg

SEQ ID NO: 165 - DNA, 56 bp, synthetic construct
  source 1..56: mol_type = other DNA
gcccttgctcaccatttaattaattcctccttttatattattcataatttagatcc

SEQ ID NO: 166 - DNA, 36 bp, synthetic construct
  source 1..36: mol_type = other DNA
agaagcttggcatagggcgcttcatgtcaacaatct

SEQ ID NO: 167 - DNA, 42 bp, synthetic construct
  source 1..42: mol_type = other DNA
gcccttgctcaccattgttttgatctcctccaataatctatg

SEQ ID NO: 168 - DNA, 711 bp, synthetic construct
  source 1..711: mol_type = other DNA
atggtgagcaagggcgaggaggataacatggccatcatcaaggagttcatgcgcttcaaggtgcacatggagggctccgtgaacggccacgagttcgagatcgagggcgagggcgagggccgcccctacgagggcacccagaccgccaagctgaaggtgaccaagggtggccccctgcccttcgcctgggacatcctgtcccctcagttcatgtacggctccaaggcctacgtgaagcaccccgccgacatccccgactacttgaagctgtccttccccgagggcttcaagtgggagcgcgtgatgaacttcgaggacggcggcgtggtgaccgtgacccaggactcctccctgcaggacggcgagttcatctacaaggtgaagctgcgcggcaccaacttcccctccgacggccccgtaatgcagaagaagaccatgggctgggaggcctcctccgagcggatgtaccccgaggacggcgccctgaagggcgagatcaagcagaggctgaagctgaaggacggcggccactacgacgctgaggtcaagaccacctacaaggccaagaagcccgtgcagctgcccggcgcctacaacgtcaacatcaagttggacatcacctcccacaacgaggactacaccatcgtggaacagtacgaacgcgccgagggccgccactccaccggcggcatggacgagctgtacaagtag

SEQ ID NO: 169 - protein, 38 aa, synthetic construct
  VARIANT 2: note = X can be any amino acid
  VARIANT 3: note = S or A
  VARIANT 4: note = V or I
  VARIANT 6: note = X can be any amino acid
  VARIANT 8: note = F or I
  VARIANT 10: note = S or A
  VARIANT 13: note = X can be any amino acid
  VARIANT 15: note = V or I
  VARIANT 16: note = X can be any amino acid
  VARIANT 17: note = X can be any amino acid
  VARIANT 19: note = V or I
  VARIANT 20: note = X can be any amino acid
  VARIANT 22: note = V or I
  VARIANT 23: note = X can be any amino acid
  VARIANT 24: note = X can be any amino acid
  VARIANT 28: note = G or N
  VARIANT 31: note = D or T
  VARIANT 32: note = X can be any amino acid
  VARIANT 33: note = I or V
  VARIANT 34: note = X can be any amino acid
  VARIANT 35: note = X can be any amino acid
  VARIANT 36: note = A or F
MXXXFXIXQXIFXGXXXLXXSXXXGAQXVFXXXXXXSS